European Patent Application EP 4 116 326 A1, published January 11, 2023. Title: MONOCLONAL AND POLYCLONAL ANTIBODY AND OXYTOCIN QUANTIFICATION METHOD BASED ON SAME. Applicant: Universidad de Murcia. Application EP21779084.9. The sequence listing filed with the application follows.

SEQUENCE LISTING (23 sequences)

SEQ ID NO: 1 - protein, 9 aa, Artificial Sequence
  Oxytocin
CYIQNCPLG

SEQ ID NO: 2 - protein, 136 aa, Artificial Sequence
  Variable domain of the heavy chain VH including signal peptide
MDWLWNLLFLMAAAQSIQAQIQLVQSGPELKKPGETVKISCKASGYIFTNYGMNWVKQAPGKNLKWMGWINTNTGEPTYAEEFKGRFAFSLETSASIAYLKINNLKNEDTATYFCSRGGLLPLSYWGQGTLVTVSA

SEQ ID NO: 3 - protein, 117 aa, Artificial Sequence
  Variable domain of the heavy chain VH
QIQLVQSGPELKKPGETVKISCKASGYIFTNYGMNWVKQAPGKNLKWMGWINTNTGEPTYAEEFKGRFAFSLETSASIAYLKINNLKNEDTATYFCSRGGLLPLSYWGQGTLVTVSA

SEQ ID NO: 4 - protein, 19 aa, Artificial Sequence
  Signal peptide of the heavy chain VH
MDWLWNLLFLMAAAQSIQA

SEQ ID NO: 5 - protein, 30 aa, Artificial Sequence
  FR1 framework region of the heavy chain VH
QIQLVQSGPELKKPGETVKISCKASGYIFT

SEQ ID NO: 6 - protein, 5 aa, Artificial Sequence
  CDR1 region of the heavy chain VH
NYGMN

SEQ ID NO: 7 - protein, 14 aa, Artificial Sequence
  FR2 framework region of the heavy chain VH
WVKQAPGKNLKWMG

SEQ ID NO: 8 - protein, 17 aa, Artificial Sequence
  CDR2 region of the heavy chain VH
WINTNTGEPTYAEEFKG

SEQ ID NO: 9 - protein, 32 aa, Artificial Sequence
  FR3 framework region of the heavy chain VH
RFAFSLETSASIAYLKINNLKNEDTATYFCSR

SEQ ID NO: 10 - protein, 8 aa, Artificial Sequence
  CDR3 region of the heavy chain VH
GGLLPLSY

SEQ ID NO: 11 - protein, 11 aa, Artificial Sequence
  FR4 framework region of the heavy chain VH
WGQGTLVTVSA

SEQ ID NO: 12 - protein, 131 aa, Artificial Sequence
  Variable domain of the light chain VL including signal peptide
MKLPVRLLVLMFWIPASTSDVVMTQTPLSLPVSLGDQASISCRSSQSLVHSNGNTYLHWFLQKPGQSPKLLIYKVSNRFSGVPDRFSGSGSGTDFTLKISRVEAEDLGVYFCSQSTHFPWTFGGGTKLEIK

SEQ ID NO: 13 - protein, 112 aa, Artificial Sequence
  Variable domain of the light chain VL
DVVMTQTPLSLPVSLGDQASISCRSSQSLVHSNGNTYLHWFLQKPGQSPKLLIYKVSNRFSGVPDRFSGSGSGTDFTLKISRVEAEDLGVYFCSQSTHFPWTFGGGTKLEIK

SEQ ID NO: 14 - protein, 19 aa, Artificial Sequence
  Signal peptide of the light chain VL
MKLPVRLLVLMFWIPASTS

SEQ ID NO: 15 - protein, 23 aa, Artificial Sequence
  FR1 framework region of the light chain VL
DVVMTQTPLSLPVSLGDQASISC

SEQ ID NO: 16 - protein, 16 aa, Artificial Sequence
  CDR1 region of the light chain VL
RSSQSLVHSNGNTYLH

SEQ ID NO: 17 - protein, 15 aa, Artificial Sequence
  FR2 framework region of the light chain VL
WFLQKPGQSPKLLIY

SEQ ID NO: 18 - protein, 7 aa, Artificial Sequence
  CDR2 region of the light chain VL
KVSNRFS

SEQ ID NO: 19 - protein, 32 aa, Artificial Sequence
  FR3 framework region of the light chain VL
GVPDRFSGSGSGTDFTLKISRVEAEDLGVYFC

SEQ ID NO: 20 - protein, 9 aa, Artificial Sequence
  CDR3 region of the light chain VL
SQSTHFPWT

SEQ ID NO: 21 - protein, 10 aa, Artificial Sequence
  FR4 framework region of the light chain VL
FGGGTKLEIK

SEQ ID NO: 22 - DNA, 408 bp, Artificial Sequence
  Nucleotide sequence encoding the variable domain of the heavy chain VH including signal peptide
atggattggctgtggaacttgctattcctgatggcagctgcccaaagtatccaagcacagatccagttggtgcagtctggacctgagctgaagaagcctggagagacagtcaagatctcctgcaaggcttctggatatatcttcacaaactatggaatgaactgggtgaagcaggctccaggaaagaatttaaagtggatgggctggataaacaccaacactggagagccaacatatgctgaagagttcaagggacggtttgccttctctttggaaacctctgccagtattgcctatttgaagatcaacaacctcaaaaatgaggacacggctacatatttctgttcaagagggggattactaccactttcttattggggccaagggactctggtcactgtctctgca

SEQ ID NO: 23 - DNA, 393 bp, Artificial Sequence
  Nucleotide sequence encoding the variable domain of the light chain VL including signal peptide
atgaagttgcctgttaggctgttggtgctgatgttctggattcctgcttccaccagtgatgttgtgatgacccaaactccactctccctgcctgtcagtcttggagatcaagcctccatctcttgcagatctagtcagagccttgtacacagtaatggaaacacctatttacattggttcctgcagaagccaggccagtctccaaagctcctgatctacaaggtttccaaccgattttctggggtcccagacaggttcagtggcagtggatcagggacagatttcacactcaagatcagcagagtggaggctgaggatctgggagtttatttctgctctcaaagtacacattttccgtggacgttcggtggaggcaccaagctggaaatcaaa